European Patent Specification EP 3 889 604 B1, published February 12, 2025. Title: SEVERE ACUTE RESPIRATORY SYNDROME (SARS) - ASSOCIATED CORONAVIRUS DIAGNOSTICS. Applicant: INSTITUT PASTEUR. The sequence listing filed with the application follows.

SEQUENCE LISTING (1 sequence)

SEQ ID NO: 1 - protein, 445 aa, Severe acute respiratory syndrome (SARS)-associated coronavirus-2 N protein
MKHHHHHHPMSDYDIPTTENLYFQGAMSDNGPQNQRNAPRITFGGPSDSTGSNQNGERSGARSKQRRPQGLPNNTASWFTALTQHGKEDLKFPRGQGVPINTNSSPDDQIGYYRRATRRIRGGDGKMKDLSPRWYFYYLGTGPEAGLPYGANKDGIIWVATEGALNTPKDHIGTRNPANNAAIVLQLPQGTTLPKGFYAEGSRGGSQASSRSSSRSRNSSRNSTPGSSRGTSPARMAGNGGDAALALLLLDRLNQLESKMSGKGQQQQGQTVTKKSAAEASKKPRQKRTATKAYNVTQAFGRRGPEQTQGNFGDQELIRQGTDYKHWPQIAQFAPSASAFFGMSRIGMEVTPSGTWLTYTGAIKLDDKDPNFKDQVILLNKHIDAYKTFPPTEPKKDKKKKADETQALPQRQKKQQTVTLLPAADLDDFSKQLQQSMSSADSTQA